European Patent Application EP 4 353 220 A1, published April 17, 2024. Title: Use of a liquid aqueous composition for solubilization and stabilization of an antibody-drug conjugate. Applicant: PIERRE FABRE MEDICAMENT. The sequence listing filed with the application follows.

SEQUENCE LISTING (82 sequences)

SEQ ID NO: 1 - protein, 8 aa, synthetic construct
  VARIANT 3: note = X is T or S
  VARIANT 8: note = X is Y or F
GYXFTSYX

SEQ ID NO: 2 - protein, 8 aa, synthetic construct
IWPGDGST

SEQ ID NO: 3 - protein, 13 aa, synthetic construct
ASPMITPNYAMDY

SEQ ID NO: 4 - protein, 6 aa, synthetic construct
  VARIANT 4: note = X is S or N
QDIXKY

SEQ ID NO: 5 - skipped

SEQ ID NO: 6 - protein, 9 aa, synthetic construct
  VARIANT 5: note = X is T or A
QQGSXLPYT

SEQ ID NO: 7 - protein, 8 aa, synthetic construct
GYTFTSYY

SEQ ID NO: 8 - protein, 8 aa, synthetic construct
GYSFTSYF

SEQ ID NO: 9 - protein, 6 aa, synthetic construct
QDISKY

SEQ ID NO: 10 - protein, 6 aa, synthetic construct
QDINKY

SEQ ID NO: 11 - protein, 9 aa, synthetic construct
QQGSTLPYT

SEQ ID NO: 12 - protein, 9 aa, synthetic construct
QQGSALPYT

SEQ ID NO: 13 - protein, 120 aa, synthetic construct
QVQLQQSGPELVKPGASVKMSCKASGYTFTSYYIYWVKQRPGQGLEWLGWIWPGDGSTKYNEKFKDKTTLTADKSSNTAYMFLSSLTSEDSAVYFCASPMITPNYAMDYWGQGASVTVSS

SEQ ID NO: 14 - protein, 120 aa, synthetic construct
QVQLQQSGPELVKPGASVKMSCKASGYTFTSYYIHWVKQRPGQGLEWIGWIWPGDGSTKYNEKFKGKTTLTADKSSSTAYMFLSSLTSEDSAVYFCASPMITPNYAMDYWGQGASVTVSS

SEQ ID NO: 15 - protein, 120 aa, synthetic construct
QVQLQQSGSELVKPGASVKLSCKASGYTFTSYYIHWVKQRPGQGLEWIGWIWPGDGSTKYNERFKGKTTLTADKSSSTAYMFLSSLTSEDSAVYFCASPMITPNYAMDYWGQGASVTVSS

SEQ ID NO: 16 - protein, 120 aa, synthetic construct
QVQLQQSGPELVKPGDSVKMSCKASGYSFTSYFIHWVKQRPGQGLEWIGWIWPGDGSTKYNEKFKGKTTLTTDKSSSTAYMFLNSLTSEDSAVYFCASPMITPNYAMDYWGQGASVTVSS

SEQ ID NO: 17 - protein, 120 aa, synthetic construct
QVQLQQSGSELVKPGASVKMSCKASGYTFTSYYIHWVKQRPGQGLEWIGWIWPGDGSTKYNERFKGKTTLTADKSSSTAYMFLSSLTSEDSAVYFCASPMITPNYAMDYWGQGASVTVSS

SEQ ID NO: 18 - protein, 107 aa, synthetic construct
DIQMTQTTSSLSASLGDRVTISCRASQDISKYLNWYQQQPDGTIKLLIYYTSRLHSGVPSRFSGRGSGTDYSLTISNVEQEDIATYFCQQGSTLPYTFGGGTKLEIK

SEQ ID NO: 19 - protein, 107 aa, synthetic construct
DIQMTQTTSSLSASLGDRVTISCRASQDINKYLNWYQQQPDGTVKLLIYYTSRLHSGVPSRFSGRGSGTDYSLTISNLEQEDIATYFCQQGSTLPYTFGGGTKLEIK

SEQ ID NO: 20 - protein, 107 aa, synthetic construct
DIQMTQTTSSLSASLGDRVTFSCRASQDISKYLNWYQQQPDGTIKLLIYYTSRLHSGVPSRFSGRGSGTDYSLTITNLEQEDIATYFCQQGSALPYTFGGGTKLEIK

SEQ ID NO: 21 - protein, 107 aa, synthetic construct
DIQMTQTTSSLSASLGDRVTISCRASQDISKYLNWYQQQPDGTVKLLIYYTSRLHSGVPSRFSGRGSGTDYSLTISNLEQEDIATYFCQQGSTLPYTFGGGTKLEIK

SEQ ID NO: 22 - protein, 107 aa, synthetic construct
DIQMTQTTSSLSASLGDRVTISCRASQDISKYLNWYQQQPDGTIKLLIYYTSRLHSGVPSRFSGRGSGTDYSLTITNLEQEDIATYFCQQGSALPYTFGGGTKLEIK

SEQ ID NO: 23 - protein, 449 aa, synthetic construct
QVQLQQSGPELVKPGASVKMSCKASGYTFTSYYIYWVKQRPGQGLEWLGWIWPGDGSTKYNEKFKDKTTLTADKSSNTAYMFLSSLTSEDSAVYFCASPMITPNYAMDYWGQGASVTVSSASTKGPSVFPLAPSSKSTSGGTAALGCLVKDYFPEPVTVSWNSGALTSGVHTFPAVLQSSGLYSLSSVVTVPSSSLGTQTYICNVNHKPSNTKVDKRVEPKSCDKTHTCPPCPAPELLGGPSVFLFPPKPKDTLMISRTPEVTCVVVDVSHEDPEVKFNWYVDGVEVHNAKTKPREEQYNSTYRVVSVLTVLHQDWLNGKEYKCKVSNKALPAPIEKTISKAKGQPREPQVYTLPPSREEMTKNQVSLTCLVKGFYPSDIAVEWESNGQPENNYKTTPPVLDSDGSFFLYSKLTVDKSRWQQGNVFSCSVMHEALHNHYTQKSLSLSPG

SEQ ID NO: 24 - protein, 449 aa, synthetic construct
QVQLQQSGPELVKPGASVKMSCKASGYTFTSYYIHWVKQRPGQGLEWIGWIWPGDGSTKYNEKFKGKTTLTADKSSSTAYMFLSSLTSEDSAVYFCASPMITPNYAMDYWGQGASVTVSSASTKGPSVFPLAPSSKSTSGGTAALGCLVKDYFPEPVTVSWNSGALTSGVHTFPAVLQSSGLYSLSSVVTVPSSSLGTQTYICNVNHKPSNTKVDKRVEPKSCDKTHTCPPCPAPELLGGPSVFLFPPKPKDTLMISRTPEVTCVVVDVSHEDPEVKFNWYVDGVEVHNAKTKPREEQYNSTYRVVSVLTVLHQDWLNGKEYKCKVSNKALPAPIEKTISKAKGQPREPQVYTLPPSREEMTKNQVSLTCLVKGFYPSDIAVEWESNGQPENNYKTTPPVLDSDGSFFLYSKLTVDKSRWQQGNVFSCSVMHEALHNHYTQKSLSLSPG

SEQ ID NO: 25 - protein, 449 aa, synthetic construct
QVQLQQSGSELVKPGASVKLSCKASGYTFTSYYIHWVKQRPGQGLEWIGWIWPGDGSTKYNERFKGKTTLTADKSSSTAYMFLSSLTSEDSAVYFCASPMITPNYAMDYWGQGASVTVSSASTKGPSVFPLAPSSKSTSGGTAALGCLVKDYFPEPVTVSWNSGALTSGVHTFPAVLQSSGLYSLSSVVTVPSSSLGTQTYICNVNHKPSNTKVDKRVEPKSCDKTHTCPPCPAPELLGGPSVFLFPPKPKDTLMISRTPEVTCVVVDVSHEDPEVKFNWYVDGVEVHNAKTKPREEQYNSTYRVVSVLTVLHQDWLNGKEYKCKVSNKALPAPIEKTISKAKGQPREPQVYTLPPSREEMTKNQVSLTCLVKGFYPSDIAVEWESNGQPENNYKTTPPVLDSDGSFFLYSKLTVDKSRWQQGNVFSCSVMHEALHNHYTQKSLSLSPG

SEQ ID NO: 26 - protein, 449 aa, synthetic construct
QVQLQQSGPELVKPGDSVKMSCKASGYSFTSYFIHWVKQRPGQGLEWIGWIWPGDGSTKYNEKFKGKTTLTTDKSSSTAYMFLNSLTSEDSAVYFCASPMITPNYAMDYWGQGASVTVSSASTKGPSVFPLAPSSKSTSGGTAALGCLVKDYFPEPVTVSWNSGALTSGVHTFPAVLQSSGLYSLSSVVTVPSSSLGTQTYICNVNHKPSNTKVDKRVEPKSCDKTHTCPPCPAPELLGGPSVFLFPPKPKDTLMISRTPEVTCVVVDVSHEDPEVKFNWYVDGVEVHNAKTKPREEQYNSTYRVVSVLTVLHQDWLNGKEYKCKVSNKALPAPIEKTISKAKGQPREPQVYTLPPSREEMTKNQVSLTCLVKGFYPSDIAVEWESNGQPENNYKTTPPVLDSDGSFFLYSKLTVDKSRWQQGNVFSCSVMHEALHNHYTQKSLSLSPG

SEQ ID NO: 27 - protein, 449 aa, synthetic construct
QVQLQQSGSELVKPGASVKMSCKASGYTFTSYYIHWVKQRPGQGLEWIGWIWPGDGSTKYNERFKGKTTLTADKSSSTAYMFLSSLTSEDSAVYFCASPMITPNYAMDYWGQGASVTVSSASTKGPSVFPLAPSSKSTSGGTAALGCLVKDYFPEPVTVSWNSGALTSGVHTFPAVLQSSGLYSLSSVVTVPSSSLGTQTYICNVNHKPSNTKVDKRVEPKSCDKTHTCPPCPAPELLGGPSVFLFPPKPKDTLMISRTPEVTCVVVDVSHEDPEVKFNWYVDGVEVHNAKTKPREEQYNSTYRVVSVLTVLHQDWLNGKEYKCKVSNKALPAPIEKTISKAKGQPREPQVYTLPPSREEMTKNQVSLTCLVKGFYPSDIAVEWESNGQPENNYKTTPPVLDSDGSFFLYSKLTVDKSRWQQGNVFSCSVMHEALHNHYTQKSLSLSPG

SEQ ID NO: 28 - protein, 214 aa, synthetic construct
DIQMTQTTSSLSASLGDRVTISCRASQDISKYLNWYQQQPDGTIKLLIYYTSRLHSGVPSRFSGRGSGTDYSLTISNVEQEDIATYFCQQGSTLPYTFGGGTKLEIKRTVAAPSVFIFPPSDEQLKSGTASVVCLLNNFYPREAKVQWKVDNALQSGNSQESVTEQDSKDSTYSLSSTLTLSKADYEKHKVYACEVTHQGLSSPVTKSFNRGEC

SEQ ID NO: 29 - protein, 214 aa, synthetic construct
DIQMTQTTSSLSASLGDRVTISCRASQDINKYLNWYQQQPDGTVKLLIYYTSRLHSGVPSRFSGRGSGTDYSLTISNLEQEDIATYFCQQGSTLPYTFGGGTKLEIKRTVAAPSVFIFPPSDEQLKSGTASVVCLLNNFYPREAKVQWKVDNALQSGNSQESVTEQDSKDSTYSLSSTLTLSKADYEKHKVYACEVTHQGLSSPVTKSFNRGEC

SEQ ID NO: 30 - protein, 214 aa, synthetic construct
DIQMTQTTSSLSASLGDRVTFSCRASQDISKYLNWYQQQPDGTIKLLIYYTSRLHSGVPSRFSGRGSGTDYSLTITNLEQEDIATYFCQQGSALPYTFGGGTKLEIKRTVAAPSVFIFPPSDEQLKSGTASVVCLLNNFYPREAKVQWKVDNALQSGNSQESVTEQDSKDSTYSLSSTLTLSKADYEKHKVYACEVTHQGLSSPVTKSFNRGEC

SEQ ID NO: 31 - protein, 214 aa, synthetic construct
DIQMTQTTSSLSASLGDRVTISCRASQDISKYLNWYQQQPDGTVKLLIYYTSRLHSGVPSRFSGRGSGTDYSLTISNLEQEDIATYFCQQGSTLPYTFGGGTKLEIKRTVAAPSVFIFPPSDEQLKSGTASVVCLLNNFYPREAKVQWKVDNALQSGNSQESVTEQDSKDSTYSLSSTLTLSKADYEKHKVYACEVTHQGLSSPVTKSFNRGEC

SEQ ID NO: 32 - protein, 214 aa, synthetic construct
DIQMTQTTSSLSASLGDRVTISCRASQDISKYLNWYQQQPDGTIKLLIYYTSRLHSGVPSRFSGRGSGTDYSLTITNLEQEDIATYFCQQGSALPYTFGGGTKLEIKRTVAAPSVFIFPPSDEQLKSGTASVVCLLNNFYPREAKVQWKVDNALQSGNSQESVTEQDSKDSTYSLSSTLTLSKADYEKHKVYACEVTHQGLSSPVTKSFNRGEC

SEQ ID NO: 33 - protein, 120 aa, synthetic construct
QVQLVQSGAEVKKPGASVKVSCKASGYTFTSYYMHWVRQAPGQGLEWMGIIWPGDGSTSYAQKFQGRVTMTRDTSTSTVYMELSSLRSEDTAVYYCASPMITPNYAMDYWGQGTLVTVSS

SEQ ID NO: 34 - protein, 120 aa, synthetic construct
QVQLVQSGAEVKKPGASVKMSCKASGYTFTSYYIYWVKQAPGQGLEWLGWIWPGDGSTKYNEKFQGRVTLTADKSSNTAYMFLSSLRSEDTAVYFCASPMITPNYAMDYWGQGTLVTVSS

SEQ ID NO: 35 - protein, 107 aa, synthetic construct
DIQMTQSPSSLSASVGDRVTITCRASQDISKYLNWYQQKPGKAPKLLIYYTSSLQSGVPSRFSGSGSGTDFTLTISSLQPEDFATYYCQQGSTLPYTFGGGTKVEIK

SEQ ID NO: 36 - protein, 107 aa, synthetic construct
DIQMTQSPSSLSASVGDRVTISCRASQDISKYLNWYQQKPGKAPKLLIYYTSRLHSGVPSRFSGRGSGTDYSLTISNLQPEDFATYFCQQGSTLPYTFGGGTKVEIK

SEQ ID NO: 37 - protein, 449 aa, synthetic construct
QVQLVQSGAEVKKPGASVKVSCKASGYTFTSYYMHWVRQAPGQGLEWMGIIWPGDGSTSYAQKFQGRVTMTRDTSTSTVYMELSSLRSEDTAVYYCASPMITPNYAMDYWGQGTLVTVSSASTKGPSVFPLAPSSKSTSGGTAALGCLVKDYFPEPVTVSWNSGALTSGVHTFPAVLQSSGLYSLSSVVTVPSSSLGTQTYICNVNHKPSNTKVDKRVEPKSCDKTHTCPPCPAPELLGGPSVFLFPPKPKDTLMISRTPEVTCVVVDVSHEDPEVKFNWYVDGVEVHNAKTKPREEQYNSTYRVVSVLTVLHQDWLNGKEYKCKVSNKALPAPIEKTISKAKGQPREPQVYTLPPSREEMTKNQVSLTCLVKGFYPSDIAVEWESNGQPENNYKTTPPVLDSDGSFFLYSKLTVDKSRWQQGNVFSCSVMHEALHNHYTQKSLSLSPG

SEQ ID NO: 38 - protein, 449 aa, synthetic construct
QVQLVQSGAEVKKPGASVKMSCKASGYTFTSYYIYWVKQAPGQGLEWLGWIWPGDGSTKYNEKFQGRVTLTADKSSNTAYMFLSSLRSEDTAVYFCASPMITPNYAMDYWGQGTLVTVSSASTKGPSVFPLAPSSKSTSGGTAALGCLVKDYFPEPVTVSWNSGALTSGVHTFPAVLQSSGLYSLSSVVTVPSSSLGTQTYICNVNHKPSNTKVDKRVEPKSCDKTHTCPPCPAPELLGGPSVFLFPPKPKDTLMISRTPEVTCVVVDVSHEDPEVKFNWYVDGVEVHNAKTKPREEQYNSTYRVVSVLTVLHQDWLNGKEYKCKVSNKALPAPIEKTISKAKGQPREPQVYTLPPSREEMTKNQVSLTCLVKGFYPSDIAVEWESNGQPENNYKTTPPVLDSDGSFFLYSKLTVDKSRWQQGNVFSCSVMHEALHNHYTQKSLSLSPG

SEQ ID NO: 39 - protein, 214 aa, synthetic construct
DIQMTQSPSSLSASVGDRVTITCRASQDISKYLNWYQQKPGKAPKLLIYYTSSLQSGVPSRFSGSGSGTDFTLTISSLQPEDFATYYCQQGSTLPYTFGGGTKVEIKRTVAAPSVFIFPPSDEQLKSGTASVVCLLNNFYPREAKVQWKVDNALQSGNSQESVTEQDSKDSTYSLSSTLTLSKADYEKHKVYACEVTHQGLSSPVTKSFNRGEC

SEQ ID NO: 40 - protein, 214 aa, synthetic construct
DIQMTQSPSSLSASVGDRVTISCRASQDISKYLNWYQQKPGKAPKLLIYYTSRLHSGVPSRFSGRGSGTDYSLTISNLQPEDFATYFCQQGSTLPYTFGGGTKVEIKRTVAAPSVFIFPPSDEQLKSGTASVVCLLNNFYPREAKVQWKVDNALQSGNSQESVTEQDSKDSTYSLSSTLTLSKADYEKHKVYACEVTHQGLSSPVTKSFNRGEC

SEQ ID NO: 41 - protein, 120 aa, synthetic construct
  VARIANT 20: note = X is M or V
  VARIANT 34: note = X is I or M
  VARIANT 35: note = Xis Y or H
  VARIANT 38: note = X is K or R
  VARIANT 48: note = X is L or M
  VARIANT 50: note = X is W or I
  VARIANT 59: note = X is K or S
  VARIANT 61: note = X is N or A
  VARIANT 70: note = X is L or M
  VARIANT 72: note = X is A or R
  VARIANT 74: note = X is K or T
  VARIANT 76: note = X is S or T
  VARIANT 77: note = X is N or S
  VARIANT 79: note = X is A or V
  VARIANT 82: note = X is F or E
  VARIANT 95: note = X is F or Y
QVQLVQSGAEVKKPGASVKXSCKASGYTFTSYYXXWVXQAPGQGLEWXGXIWPGDGSTXYXZKFQGRVTXTXDXSXXTXYMXLSSLRSEDTAVYXCASPMITPNYAMDYWGQGTLVTVSS

SEQ ID NO: 42 - protein, 107 aa, synthetic construct
  VARIANT 22: note = X is S or T
  VARIANT 53: note = X is R or S
  VARIANT 55: note = X is H or Q
  VARIANT 64: note = X is R or S
  VARIANT 70: note = X is Y or F
  VARIANT 71: note = X is S or T
  VARIANT 76: note = X is N or S
  VARIANT 86: note = X is F or Y
DIQMTQSPSSLSASVGDRVTIXCRASQDISKYLNWYQQKPGKAPKLLIYYTSXLXSGVPSRFSGXGSGTDXXLTISXLQPEDFATYXCQQGSTLPYTFGGGTKVEIK

SEQ ID NO: 43 - protein, 329 aa, synthetic construct
ASTKGPSVFPLAPSSKSTSGGTAALGCLVKDYFPEPVTVSWNSGALTSGVHTFPAVLQSSGLYSLSSVVTVPSSSLGTQTYICNVNHKPSNTKVDKRVEPKSCDKTHTCPPCPAPELLGGPSVFLFPPKPKDTLMISRTPEVTCVVVDVSHEDPEVKFNWYVDGVEVHNAKTKPREEQYNSTYRVVSVLTVLHQDWLNGKEYKCKVSNKALPAPIEKTISKAKGQPREPQVYTLPPSREEMTKNQVSLTCLVKGFYPSDIAVEWESNGQPENNYKTTPPVLDSDGSFFLYSKLTVDKSRWQQGNVFSCSVMHEALHNHYTQKSLSLSPG

SEQ ID NO: 44 - protein, 326 aa, synthetic construct
ASTKGPSVFPLAPCSRSTSESTAALGCLVKDYFPEPVTVSWNSGALTSGVHTFPAVLQSSGLYSLSSVVTVPSSSLGTKTYTCNVDHKPSNTKVDKRVESKYGPPCPPCPAPEFLGGPSVFLFPPKPKDTLMISRTPEVTCVVVDVSQEDPEVQFNWYVDGVEVHNAKTKPREEQFNSTYRVVSVLTVLHQDWLNGKEYKCKVSNKGLPSSIEKTISKAKGQPREPQVYTLPPSQEEMTKNQVSLTCLVKGFYPSDIAVEWESNGQPENNYKTTPPVLDSDGSFFLYSRLTVDKSRWQEGNVFSCSVMHEALHNHYTQKSLSLSLG

SEQ ID NO: 45 - protein, 107 aa, synthetic construct [sequence omitted]

SEQ ID NO: 46 - protein, 98 aa, synthetic construct
QVQLVQSGAEVKKPGASVKVSCKASGYTFTSYYMHWVRQAPGQGLEWMGIINPSGGSTSYAQKFQGRVTMTRDTSTSTVYMELSSLRSEDTAVYYCAR

SEQ ID NO: 47 - protein, 95 aa, synthetic construct
DIQMTQSPSSLSASVGDRVTITCRASQSISSYLNWYQQKPGKAPKLLIYAASSLQSGVPSRFSGSGSGTDFTLTISSLQPEDFATYYCQQSYSTP

SEQ ID NO: 48 - protein, 15 aa, synthetic construct
YFDYWGQGTLVTVSS

SEQ ID NO: 49 - protein, 12 aa, synthetic construct
LTFGGGTKVEIK

SEQ ID NO: 50 - protein, 1367 aa, synthetic construct
MKSGSGGGSPTSLWGLLFLSAALSLWPTSGEICGPGIDIRNDYQQLKRLENCTVIEGYLHILLISKAEDYRSYRFPKLTVITEYLLLFRVAGLESLGDLFPNLTVIRGWKLFYNYALVIFEMTNLKDIGLYNLRNITRGAIRIEKNADLCYLSTVDWSLILDAVSNNYIVGNKPPKECGDLCPGTMEEKPMCEKTTINNEYNYRCWTTNRCQKMCPSTCGKRACTENNECCHPECLGSCSAPDNDTACVACRHYYYAGVCVPACPPNTYRFEGWRCVDRDFCANILSAESSDSEGFVIHDGECMQECPSGFIRNGSQSMYCIPCEGPCPKVCEEEKKTKTIDSVTSAQMLQGCTIFKGNLLINIRRGNNIASELENFMGLIEVVTGYVKIRHSHALVSLSFLKNLRLILGEEQLEGNYSFYVLDNQNLQQLWDWDHRNLTIKAGKMYFAFNPKLCVSEIYRMEEVTGTKGRQSKGDINTRNNGERASCESDVLHFTSTTTSKNRIIITWHRYRPPDYRDLISFTVYYKEAPFKNVTEYDGQDACGSNSWNMVDVDLPPNKDVEPGILLHGLKPWTQYAVYVKAVTLTMVENDHIRGAKSEILYIRTNASVPSIPLDVLSASNSSSQLIVKWNPPSLPNGNLSYYIVRWQRQPQDGYLYRHNYCSKDKIPIRKYADGTIDIEEVTENPKTEVCGGEKGPCCACPKTEAEKQAEKEEAEYRKVFENFLHNSIFVPRPERKRRDVMQVANTTMSSRSRNTTAADTYNITDPEELETEYPFFESRVDNKERTVISNLRPFTLYRIDIHSCNHEAEKLGCSASNFVFARTMPAEGADDIPGPVTWEPRPENSIFLKWPEPENPNGLILMYEIKYGSQVEDQRECVSRQEYRKYGGAKLNRLNPGNYTARIQATSLSGNGSWTDPVFFYVQAKTGYENFIHLIIALPVAVLLIVGGLVIMLYVFHRKRNNSRLGNGVLYASVNPEYFSAADVYVPDEWEVAREKITMSRELGQGSFGMVYEGVAKGVVKDEPETRVAIKTVNEAASMRERIEFLNEASVMKEFNCHHVVRLLGVVSQGQPTLVIMELMTRGDLKSYLRSLRPEMENNPVLAPPSLSKMIQMAGEIADGMAYLNANKFVHRDLAARNCMVAEDFTVKIGDFGMTRDIYETDYYRKGGKGLLPVRWMSPESLKDGVFTTYSDVWSFGVVLWEIATLAEQPYQGLSNEQVLRFVMEGGLLDKPDNCPDMLFELMRMCWQYNPKMRPSFLEIISSIKEEMEPGFREVSFYYSEENKLPEPEELDLEPENMESVPLDPSASSSSLPLPDRHSGHKAENGPGPGVLVLRASFDERQPYAHMNGGRKNERALPLPQSSTC

SEQ ID NO: 51 - protein, 932 aa, synthetic construct
MKSGSGGGSPTSLWGLLFLSAALSLWPTSGEICGPGIDIRNDYQQLKRLENCTVIEGYLHILLISKAEDYRSYRFPKLTVITEYLLLFRVAGLESLGDLFPNLTVIRGWKLFYNYALVIFEMTNLKDIGLYNLRNITRGAIRIEKNADLCYLSTVDWSLILDAVSNNYIVGNKPPKECGDLCPGTMEEKPMCEKTTINNEYNYRCWTTNRCQKMCPSTCGKRACTENNECCHPECLGSCSAPDNDTACVACRHYYYAGVCVPACPPNTYRFEGWRCVDRDFCANILSAESSDSEGFVIHDGECMQECPSGFIRNGSQSMYCIPCEGPCPKVCEEEKKTKTIDSVTSAQMLQGCTIFKGNLLINIRRGNNIASELENFMGLIEVVTGYVKIRHSHALVSLSFLKNLRLILGEEQLEGNYSFYVLDNQNLQQLWDWDHRNLTIKAGKMYFAFNPKLCVSEIYRMEEVTGTKGRQSKGDINTRNNGERASCESDVLHFTSTTTSKNRIIITWHRYRPPDYRDLISFTVYYKEAPFKNVTEYDGQDACGSNSWNMVDVDLPPNKDVEPGILLHGLKPWTQYAVYVKAVTLTMVENDHIRGAKSEILYIRTNASVPSIPLDVLSASNSSSQLIVKWNPPSLPNGNLSYYIVRWQRQPQDGYLYRHNYCSKDKIPIRKYADGTIDIEEVTENPKTEVCGGEKGPCCACPKTEAEKQAEKEEAEYRKVFENFLHNSIFVPRPERKRRDVMQVANTTMSSRSRNTTAADTYNITDPEELETEYPFFESRVDNKERTVISNLRPFTLYRIDIHSCNHEAEKLGCSASNFVFARTMPAEGADDIPGPVTWEPRPENSIFLKWPEPENPNGLILMYEIKYGSQVEDQRECVSRQEYRKYGGAKLNRLNPGNYTARIQATSLSGNGSWTDPVFFYVQAKTGYEN

SEQ ID NO: 52 - protein, 512 aa, synthetic construct
MKSGSGGGSPTSLWGLLFLSAALSLWPTSGEICGPGIDIRNDYQQLKRLENCTVIEGYLHILLISKAEDYRSYRFPKLTVITEYLLLFRVAGLESLGDLFPNLTVIRGWKLFYNYALVIFEMTNLKDIGLYNLRNITRGAIRIEKNADLCYLSTVDWSLILDAVSNNYIVGNKPPKECGDLCPGTMEEKPMCEKTTINNEYNYRCWTTNRCQKMCPSTCGKRACTENNECCHPECLGSCSAPDNDTACVACRHYYYAGVCVPACPPNTYRFEGWRCVDRDFCANILSAESSDSEGFVIHDGECMQECPSGFIRNGSQSMYCIPCEGPCPKVCEEEKKTKTIDSVTSAQMLQGCTIFKGNLLINIRRGNNIASELENFMGLIEVVTGYVKIRHSHALVSLSFLKNLRLILGEEQLEGNYSFYVLDNQNLQQLWDWDHRNLTIKAGKMYFAFNPKLCVSEIYRMEEVTGTKGRQSKGDINTRNNGERASCESDVLHFTSTTTSKNRIIITWHRY

SEQ ID NO: 53 - protein, 449 aa, synthetic construct
QVQLVQSGAEVKKPGASVKVSCKASGYTFTSYYIHWVRQAPGQGLEWMGWIWPGDGSTKYAQKFQGRVTMTRDTSTSTVYMELSSLRSEDTAVYYCASPMITPNYAMDYWGQGTLVTVSSASTKGPSVFPLAPSSKSTSGGTAALGCLVKDYFPEPVTVSWNSGALTSGVHTFPAVLQSSGLYSLSSVVTVPSSSLGTQTYICNVNHKPSNTKVDKRVEPKSCDKTHTCPPCPAPELLGGPSVFLFPPKPKDTLMISRTPEVTCVVVDVSHEDPEVKFNWYVDGVEVHNAKTKPREEQYNSTYRVVSVLTVLHQDWLNGKEYKCKVSNKALPAPIEKTISKAKGQPREPQVYTLPPSREEMTKNQVSLTCLVKGFYPSDIAVEWESNGQPENNYKTTPPVLDSDGSFFLYSKLTVDKSRWQQGNVFSCSVMHEALHNHYTQKSLSLSPG

SEQ ID NO: 54 - protein, 120 aa, synthetic construct
QVQLVQSGAEVKKPGASVKVSCKASGYTFTSYYIHWVRQAPGQGLEWMGWIWPGDGSTKYAQKFQGRVTMTRDTSTSTVYMELSSLRSEDTAVYFCASPMITPNYAMDYWGQGTLVTVSS

SEQ ID NO: 55 - protein, 449 aa, synthetic construct
QVQLVQSGAEVKKPGASVKVSCKASGYTFTSYYIHWVRQAPGQGLEWMGWIWPGDGSTKYAQKFQGRVTMTRDTSTSTVYMELSSLRSEDTAVYFCASPMITPNYAMDYWGQGTLVTVSSASTKGPSVFPLAPSSKSTSGGTAALGCLVKDYFPEPVTVSWNSGALTSGVHTFPAVLQSSGLYSLSSVVTVPSSSLGTQTYICNVNHKPSNTKVDKRVEPKSCDKTHTCPPCPAPELLGGPSVFLFPPKPKDTLMISRTPEVTCVVVDVSHEDPEVKFNWYVDGVEVHNAKTKPREEQYNSTYRVVSVLTVLHQDWLNGKEYKCKVSNKALPAPIEKTISKAKGQPREPQVYTLPPSREEMTKNQVSLTCLVKGFYPSDIAVEWESNGQPENNYKTTPPVLDSDGSFFLYSKLTVDKSRWQQGNVFSCSVMHEALHNHYTQKSLSLSPG

SEQ ID NO: 56 - protein, 120 aa, synthetic construct
QVQLVQSGAEVKKPGASVKVSCKASGYTFTSYYMHWVRQAPGQGLEWMGWIWPGDGSTKYAQKFQGRVTMTRDKSSSTVYMELSSLRSEDTAVYFCASPMITPNYAMDYWGQGTLVTVSS

SEQ ID NO: 57 - protein, 107 aa, synthetic construct
DIQMTQSPSSLSASVGDRVTITCRASQDISKYLNWYQQKPGKAPKLLIYYTSRLQSGVPSRFSGRGSGTDYSLTISSLQPEDFATYFCQQGSTLPYTFGGGTKVEIK

SEQ ID NO: 58 - protein, 449 aa, synthetic construct
QVQLVQSGAEVKKPGASVKVSCKASGYTFTSYYMHWVRQAPGQGLEWMGWIWPGDGSTKYAQKFQGRVTMTRDKSSSTVYMELSSLRSEDTAVYFCASPMITPNYAMDYWGQGTLVTVSSASTKGPSVFPLAPSSKSTSGGTAALGCLVKDYFPEPVTVSWNSGALTSGVHTFPAVLQSSGLYSLSSVVTVPSSSLGTQTYICNVNHKPSNTKVDKRVEPKSCDKTHTCPPCPAPELLGGPSVFLFPPKPKDTLMISRTPEVTCVVVDVSHEDPEVKFNWYVDGVEVHNAKTKPREEQYNSTYRVVSVLTVLHQDWLNGKEYKCKVSNKALPAPIEKTISKAKGQPREPQVYTLPPSREEMTKNQVSLTCLVKGFYPSDIAVEWESNGQPENNYKTTPPVLDSDGSFFLYSKLTVDKSRWQQGNVFSCSVMHEALHNHYTQKSLSLSPG

SEQ ID NO: 59 - protein, 214 aa, synthetic construct
DIQMTQSPSSLSASVGDRVTITCRASQDISKYLNWYQQKPGKAPKLLIYYTSRLQSGVPSRFSGRGSGTDYSLTISSLQPEDFATYFCQQGSTLPYTFGGGTKVEIKRTVAAPSVFIFPPSDEQLKSGTASVVCLLNNFYPREAKVQWKVDNALQSGNSQESVTEQDSKDSTYSLSSTLTLSKADYEKHKVYACEVTHQGLSSPVTKSFNRGEC

SEQ ID NO: 60 - protein, 107 aa, synthetic construct
DIQMTQSPSSLSASVGDRVTITCRASQDISKYLNWYQQKPGKAPKLLIYYTSRLHSGVPSRFSGRGSGTDFSLTISSLQPEDFATYFCQQGSTLPYTFGGGTKVEIK

SEQ ID NO: 61 - protein, 214 aa, synthetic construct
DIQMTQSPSSLSASVGDRVTITCRASQDISKYLNWYQQKPGKAPKLLIYYTSRLHSGVPSRFSGRGSGTDFSLTISSLQPEDFATYFCQQGSTLPYTFGGGTKVEIKRTVAAPSVFIFPPSDEQLKSGTASVVCLLNNFYPREAKVQWKVDNALQSGNSQESVTEQDSKDSTYSLSSTLTLSKADYEKHKVYACEVTHQGLSSPVTKSFNRGEC

SEQ ID NO: 62 - protein, 120 aa, synthetic construct
QVQLVQSGAEVKKPGASVKVSCKASGYTFTSYYIHWVRQAPGQGLEWMGWIWPGDGSTKYAQKFQGRVTMTRDTSSNTVYMELSSLRSEDTAVYYCASPMITPNYAMDYWGQGTLVTVSS

SEQ ID NO: 63 - protein, 449 aa, synthetic construct
QVQLVQSGAEVKKPGASVKVSCKASGYTFTSYYIHWVRQAPGQGLEWMGWIWPGDGSTKYAQKFQGRVTMTRDTSSNTVYMELSSLRSEDTAVYYCASPMITPNYAMDYWGQGTLVTVSSASTKGPSVFPLAPSSKSTSGGTAALGCLVKDYFPEPVTVSWNSGALTSGVHTFPAVLQSSGLYSLSSVVTVPSSSLGTQTYICNVNHKPSNTKVDKRVEPKSCDKTHTCPPCPAPELLGGPSVFLFPPKPKDTLMISRTPEVTCVVVDVSHEDPEVKFNWYVDGVEVHNAKTKPREEQYNSTYRVVSVLTVLHQDWLNGKEYKCKVSNKALPAPIEKTISKAKGQPREPQVYTLPPSREEMTKNQVSLTCLVKGFYPSDIAVEWESNGQPENNYKTTPPVLDSDGSFFLYSKLTVDKSRWQQGNVFSCSVMHEALHNHYTQKSLSLSPG

SEQ ID NO: 64 - protein, 120 aa, synthetic construct
QVQLVQSGAEVKKPGASVKVSCKASGYTFTSYYMHWVRQAPGQGLEWMGWIWPGDGSTKYAQKFQGRVTMTRDKSSSTVYMELSSLRSEDTAVYYCASPMITPNYAMDYWGQGTLVTVSS

SEQ ID NO: 65 - protein, 449 aa, synthetic construct
QVQLVQSGAEVKKPGASVKVSCKASGYTFTSYYMHWVRQAPGQGLEWMGWIWPGDGSTKYAQKFQGRVTMTRDKSSSTVYMELSSLRSEDTAVYYCASPMITPNYAMDYWGQGTLVTVSSASTKGPSVFPLAPSSKSTSGGTAALGCLVKDYFPEPVTVSWNSGALTSGVHTFPAVLQSSGLYSLSSVVTVPSSSLGTQTYICNVNHKPSNTKVDKRVEPKSCDKTHTCPPCPAPELLGGPSVFLFPPKPKDTLMISRTPEVTCVVVDVSHEDPEVKFNWYVDGVEVHNAKTKPREEQYNSTYRVVSVLTVLHQDWLNGKEYKCKVSNKALPAPIEKTISKAKGQPREPQVYTLPPSREEMTKNQVSLTCLVKGFYPSDIAVEWESNGQPENNYKTTPPVLDSDGSFFLYSKLTVDKSRWQQGNVFSCSVMHEALHNHYTQKSLSLSPG

SEQ ID NO: 66 - protein, 120 aa, synthetic construct
QVQLVQSGAEVKKPGASVKVSCKASGYTFTSYYMHWVRQAPGQGLEWMGWIWPGDGSTKYAQKFQGRVTMTRDTSSNTVYMELSSLRSEDTAVYFCASPMITPNYAMDYWGQGTLVTVSS

SEQ ID NO: 67 - protein, 449 aa, synthetic construct
QVQLVQSGAEVKKPGASVKVSCKASGYTFTSYYMHWVRQAPGQGLEWMGWIWPGDGSTKYAQKFQGRVTMTRDTSSNTVYMELSSLRSEDTAVYFCASPMITPNYAMDYWGQGTLVTVSSASTKGPSVFPLAPSSKSTSGGTAALGCLVKDYFPEPVTVSWNSGALTSGVHTFPAVLQSSGLYSLSSVVTVPSSSLGTQTYICNVNHKPSNTKVDKRVEPKSCDKTHTCPPCPAPELLGGPSVFLFPPKPKDTLMISRTPEVTCVVVDVSHEDPEVKFNWYVDGVEVHNAKTKPREEQYNSTYRVVSVLTVLHQDWLNGKEYKCKVSNKALPAPIEKTISKAKGQPREPQVYTLPPSREEMTKNQVSLTCLVKGFYPSDIAVEWESNGQPENNYKTTPPVLDSDGSFFLYSKLTVDKSRWQQGNVFSCSVMHEALHNHYTQKSLSLSPG

SEQ ID NO: 68 - protein, 120 aa, synthetic construct
QVQLVQSGAEVKKPGASVKVSCKASGYTFTSYYMHWVRQAPGQGLEWMGWIWPGDGSTKYAQKFQGRVTMTRDTSTSTVYMELSSLRSEDTAVYFCASPMITPNYAMDYWGQGTLVTVSS

SEQ ID NO: 69 - protein, 449 aa, synthetic construct
QVQLVQSGAEVKKPGASVKVSCKASGYTFTSYYMHWVRQAPGQGLEWMGWIWPGDGSTKYAQKFQGRVTMTRDTSTSTVYMELSSLRSEDTAVYFCASPMITPNYAMDYWGQGTLVTVSSASTKGPSVFPLAPSSKSTSGGTAALGCLVKDYFPEPVTVSWNSGALTSGVHTFPAVLQSSGLYSLSSVVTVPSSSLGTQTYICNVNHKPSNTKVDKRVEPKSCDKTHTCPPCPAPELLGGPSVFLFPPKPKDTLMISRTPEVTCVVVDVSHEDPEVKFNWYVDGVEVHNAKTKPREEQYNSTYRVVSVLTVLHQDWLNGKEYKCKVSNKALPAPIEKTISKAKGQPREPQVYTLPPSREEMTKNQVSLTCLVKGFYPSDIAVEWESNGQPENNYKTTPPVLDSDGSFFLYSKLTVDKSRWQQGNVFSCSVMHEALHNHYTQKSLSLSPG

SEQ ID NO: 70 - protein, 120 aa, synthetic construct
QVQLVQSGAEVKKPGASVKVSCKASGYTFTSYYIHWVRQAPGQGLEWMGWIWPGDGSTKYAQKFQGRVTMTRDKSTNTVYMELSSLRSEDTAVYYCASPMITPNYAMDYWGQGTLVTVSS

SEQ ID NO: 71 - protein, 449 aa, synthetic construct
QVQLVQSGAEVKKPGASVKVSCKASGYTFTSYYIHWVRQAPGQGLEWMGWIWPGDGSTKYAQKFQGRVTMTRDKSTNTVYMELSSLRSEDTAVYYCASPMITPNYAMDYWGQGTLVTVSSASTKGPSVFPLAPSSKSTSGGTAALGCLVKDYFPEPVTVSWNSGALTSGVHTFPAVLQSSGLYSLSSVVTVPSSSLGTQTYICNVNHKPSNTKVDKRVEPKSCDKTHTCPPCPAPELLGGPSVFLFPPKPKDTLMISRTPEVTCVVVDVSHEDPEVKFNWYVDGVEVHNAKTKPREEQYNSTYRVVSVLTVLHQDWLNGKEYKCKVSNKALPAPIEKTISKAKGQPREPQVYTLPPSREEMTKNQVSLTCLVKGFYPSDIAVEWESNGQPENNYKTTPPVLDSDGSFFLYSKLTVDKSRWQQGNVFSCSVMHEALHNHYTQKSLSLSPG

SEQ ID NO: 72 - protein, 120 aa, synthetic construct
QVQLVQSGAEVKKPGASVKVSCKASGYTFTSYYMHWVRQAPGQGLEWMGWIWPGDGSTKYAQKFQGRVTMTRDTSTNTVYMELSSLRSEDTAVYFCASPMITPNYAMDYWGQGTLVTVSS

SEQ ID NO: 73 - protein, 449 aa, synthetic construct
QVQLVQSGAEVKKPGASVKVSCKASGYTFTSYYMHWVRQAPGQGLEWMGWIWPGDGSTKYAQKFQGRVTMTRDTSTNTVYMELSSLRSEDTAVYFCASPMITPNYAMDYWGQGTLVTVSSASTKGPSVFPLAPSSKSTSGGTAALGCLVKDYFPEPVTVSWNSGALTSGVHTFPAVLQSSGLYSLSSVVTVPSSSLGTQTYICNVNHKPSNTKVDKRVEPKSCDKTHTCPPCPAPELLGGPSVFLFPPKPKDTLMISRTPEVTCVVVDVSHEDPEVKFNWYVDGVEVHNAKTKPREEQYNSTYRVVSVLTVLHQDWLNGKEYKCKVSNKALPAPIEKTISKAKGQPREPQVYTLPPSREEMTKNQVSLTCLVKGFYPSDIAVEWESNGQPENNYKTTPPVLDSDGSFFLYSKLTVDKSRWQQGNVFSCSVMHEALHNHYTQKSLSLSPG

SEQ ID NO: 74 - protein, 120 aa, synthetic construct
QVQLVQSGAEVKKPGASVKVSCKASGYTFTSYYMHWVRQAPGQGLEWMGWIWPGDGSTKYAQKFQGRVTMTRDTSTSTVYMELSSLRSEDTAVYYCASPMITPNYAMDYWGQGTLVTVSS

SEQ ID NO: 75 - protein, 449 aa, synthetic construct
QVQLVQSGAEVKKPGASVKVSCKASGYTFTSYYMHWVRQAPGQGLEWMGWIWPGDGSTKYAQKFQGRVTMTRDTSTSTVYMELSSLRSEDTAVYYCASPMITPNYAMDYWGQGTLVTVSSASTKGPSVFPLAPSSKSTSGGTAALGCLVKDYFPEPVTVSWNSGALTSGVHTFPAVLQSSGLYSLSSVVTVPSSSLGTQTYICNVNHKPSNTKVDKRVEPKSCDKTHTCPPCPAPELLGGPSVFLFPPKPKDTLMISRTPEVTCVVVDVSHEDPEVKFNWYVDGVEVHNAKTKPREEQYNSTYRVVSVLTVLHQDWLNGKEYKCKVSNKALPAPIEKTISKAKGQPREPQVYTLPPSREEMTKNQVSLTCLVKGFYPSDIAVEWESNGQPENNYKTTPPVLDSDGSFFLYSKLTVDKSRWQQGNVFSCSVMHEALHNHYTQKSLSLSPG

SEQ ID NO: 76 - protein, 120 aa, synthetic construct
QVQLVQSGAEVKKPGASVKVSCKASGYTFTSYYMHWVRQAPGQGLEWMGWIWPGDGSTKYAQKFQGRVTMTRDTSTNTVYMELSSLRSEDTAVYYCASPMITPNYAMDYWGQGTLVTVSS

SEQ ID NO: 77 - protein, 449 aa, synthetic construct
QVQLVQSGAEVKKPGASVKVSCKASGYTFTSYYMHWVRQAPGQGLEWMGWIWPGDGSTKYAQKFQGRVTMTRDTSTNTVYMELSSLRSEDTAVYYCASPMITPNYAMDYWGQGTLVTVSSASTKGPSVFPLAPSSKSTSGGTAALGCLVKDYFPEPVTVSWNSGALTSGVHTFPAVLQSSGLYSLSSVVTVPSSSLGTQTYICNVNHKPSNTKVDKRVEPKSCDKTHTCPPCPAPELLGGPSVFLFPPKPKDTLMISRTPEVTCVVVDVSHEDPEVKFNWYVDGVEVHNAKTKPREEQYNSTYRVVSVLTVLHQDWLNGKEYKCKVSNKALPAPIEKTISKAKGQPREPQVYTLPPSREEMTKNQVSLTCLVKGFYPSDIAVEWESNGQPENNYKTTPPVLDSDGSFFLYSKLTVDKSRWQQGNVFSCSVMHEALHNHYTQKSLSLSPG

SEQ ID NO: 78 - protein, 120 aa, synthetic construct
QVQLVQSGAEVKKPGASVKVSCKASGYTFTSYYIHWVRQAPGQGLEWMGWIWPGDGSTKYAQKFQGRVTMTRDTSTSTVYMELSSLRSEDTAVYYCASPMITPNYAMDYWGQGTLVTVSS

SEQ ID NO: 79 - protein, 4 aa, synthetic construct
GFLG

SEQ ID NO: 80 - protein, 4 aa, synthetic construct
ALAL

SEQ ID NO: 81 - protein, 4 aa, synthetic construct
GGFG

SEQ ID NO: 82 - protein, 5 aa, synthetic construct
PVGVV